European Patent Application EP 4 659 593 A1, published December 10, 2025. Title: MONASCUS PILOSUS STRAIN, COMPOSITION FOR LOSING WEIGHT AND IMPROVING GUT MICROBIOTA COMPOSITION AND USE OF SAID MONASCUS PILOSUS. Applicant: SUNWAY BIOTECH CO., LTD. Application EP. The sequence listing filed with the application follows.

SEQUENCE LISTING (14 sequences)

SEQ ID NO: 1 - DNA, 19 bp, synthetic construct
  source 1..19: mol_type = other DNA
tccgtaggtgaacctgcgg

SEQ ID NO: 2 - DNA, 20 bp, synthetic construct
  source 1..20: mol_type = other DNA
tcctccgcttattgatatgc

SEQ ID NO: 3 - DNA, 17 bp, synthetic construct
  source 1..17: mol_type = other DNA
caagatccgtgaggagt

SEQ ID NO: 4 - DNA, 21 bp, synthetic construct
  source 1..21: mol_type = other DNA
gtgaactccatctcgtccata

SEQ ID NO: 5 - DNA, 19 bp, synthetic construct
  source 1..19: mol_type = other DNA
cccaagtgctcgatccttt

SEQ ID NO: 6 - DNA, 20 bp, synthetic construct
  source 1..20: mol_type = other DNA
cctgggaggggtcgtattca

SEQ ID NO: 7 - DNA, 21 bp, synthetic construct
  source 1..21: mol_type = other DNA
cgtgccgctttgatcttttgg

SEQ ID NO: 8 - DNA, 17 bp, synthetic construct
  source 1..17: mol_type = other DNA
aggggagttggtgggca

SEQ ID NO: 9 - DNA, 22 bp, synthetic construct
  source 1..22: mol_type = other DNA
cctcacgagcatcaaaagcaaa

SEQ ID NO: 10 - DNA, 22 bp, synthetic construct
  source 1..22: mol_type = other DNA
ttggttatcaagacgcatccca

SEQ ID NO: 11 - DNA, 20 bp, synthetic construct
  source 1..20: mol_type = other DNA
agrgttygatymtggctcag

SEQ ID NO: 12 - DNA, 19 bp, synthetic construct
  source 1..19: mol_type = other DNA
rgytaccttgttacgactt

SEQ ID NO: 13 - DNA, 14 bp, synthetic construct
  source 1..14: mol_type = other DNA
cctacgggnggcwg

SEQ ID NO: 14 - DNA, 21 bp, synthetic construct
  source 1..21: mol_type = other DNA
gactachvgggtatctaatcc